European Patent Application EP 4 252 769 A2, published October 4, 2023. Title: ANTI-COMPLEMENT FACTOR C1Q ANTIBODIES AND USES THEREOF. Applicant: Annexon, Inc. The sequence listing filed with the application follows.

SEQUENCE LISTING (26 sequences)

SEQ ID NO: 1 - protein, 245 aa, Homo sapiens
MEGPRGWLVLCVLAISLASMVTEDLCRAPDGKKGEAGRPGRRGRPGLKGEQGEPGAPGIRTGIQGLKGDQGEPGPSGNPGKVGYPGPSGPLGARGIPGIKGTKGSPGNIKDQPRPAFSAIRRNPPMGGNVVIFDTVITNQEEPYQNHSGRFVCTVPGYYYFTFQVLSQWEICLSIVSSSRGQVRRSLGFCDTTNKGLFQVVSGGMVLQLQQGDQVWVEKDPKKGHIYQGSEADSVFSGFLIFPSA

SEQ ID NO: 2 - protein, 253 aa, Homo sapiens
MMMKIPWGSIPVLMLLLLLGLIDISQAQLSCTGPPAIPGIPGIPGTPGPDGQPGTPGIKGEKGLPGLAGDHGEFGEKGDPGIPGNPGKVGPKGPMGPKGGPGAPGAPGPKGESGDYKATQKIAFSATRTINVPLRRDQTIRFDHVITNMNNNYEPRSGKFTCKVPGLYYFTYHASSRGNLCVNLMRGRERAQKVVTFCDYAYNTFQVTTGGMVLKLEQGENVFLQATDKNSLLGMEGANSIFSGFLLFPDMEA

SEQ ID NO: 3 - protein, 245 aa, Homo sapiens
MDVGPSSLPHLGLKLLLLLLLLPLRGQANTGCYGIPGMPGLPGAPGKDGYDGLPGPKGEPGIPAIPGIRGPKGQKGEPGLPGHPGKNGPMGPPGMPGVPGPMGIPGEPGEEGRYKQKFQSVFTVTRQTHQPPAPNSLIRFNAVLTNPQGDYDTSTGKFTCKVPGLYYFVYHASHTANLCVLLYRSGVKVVTFCGHTSKTNQVNSGGVLLRLQVGEEVWLAVNDYYDMVGIQGSDSVFSGFLLFPD

SEQ ID NO: 4 - protein, 107 aa, Homo sapiens
DVQITQSPSYLAASPGETITINCRASKSINKYLAWYQEKPGKTNKLLIYSGSTLQSGIPSRFSGSGSGTDFTLTISSLEPEDFAMYYCQQHNEYPLTFGAGTKLELK

SEQ ID NO: 5 - protein, 11 aa, Homo sapiens
RASKSINKYLA

SEQ ID NO: 6 - protein, 7 aa, Homo sapiens
SGSTLQS

SEQ ID NO: 7 - protein, 9 aa, Homo sapiens
QQHNEYPLT

SEQ ID NO: 8 - protein, 121 aa, Homo sapiens
QVQLQQPGAELVKPGASVKLSCKSSGYHFTSYWMHWVKQRPGQGLEWIGVIHPNSGSINYNEKFESKATLTVDKSSSTAYMQLSSLTSEDSAVYYCAGERDSTEVLPMDYWGQGTSVTVSS

SEQ ID NO: 9 - protein, 10 aa, Homo sapiens
GYHFTSYWMH

SEQ ID NO: 10 - protein, 17 aa, Homo sapiens
VIHPNSGSINYNEKFES

SEQ ID NO: 11 - protein, 12 aa, Homo sapiens
ERDSTEVLPMDY

SEQ ID NO: 12 - protein, 321 aa, Homo sapiens
GATGTCCAGATAACCCAGTCTCCATCTTATCTTGCTGCATCTCCTGGAGAAACCATTACTATTAATTGCAGGGCAAGTAAGAGCATTAACAAATATTTAGCCTGGTATCAAGAGAAACCTGGGAAAACTAATAAGCTTCTTATCTACTCTGGATCCACTTTGCAATCTGGAATTCCATCAAGGTTCAGTGGCAGTGGATCTGGTACAGATTTCACTCTCACCATCAGTAGCCTGGAGCCTGAAGATTTTGCAATGTATTACTGTCAACAACATAATGAATACCCGCTCACGTTCGGTGCTGGGACCAAGCTGGAGCTGAAA

SEQ ID NO: 13 - protein, 363 aa, Homo sapiens
CAGGTCCAACTGCAGCAGCCTGGGGCTGAGCTGGTAAAGCCTGGGGCTTCAGTGAAGTTGTCCTGCAAGTCTTCTGGCTACCATTTCACCAGCTACTGGATGCACTGGGTGAAGCAGAGGCCTGGACAAGGCCTTGAGTGGATTGGAGTGATTCATCCTAATAGTGGTAGTATTAACTACAATGAGAAGTTCGAGAGCAAGGCCACACTGACTGTAGACAAATCCTCCAGCACAGCCTACATGCAACTCAGCAGCCTGACATCTGAGGACTCGGCGGTCTATTATTGTGCAGGAGAGAGAGATTCTACGGAGGTTCTCCCTATGGACTACTGGGGTCAAGGAACCTCAGTCACCGTCTCCTCA

SEQ ID NO: 14 - protein, 245 aa, Mus musculus
METSQGWLVACVLTMTLVWTVAEDVCRAPNGKDGAPGNPGRPGRPGLKGERGEPGAAGIRTGIRGFKGDPGESGPPGKPGNVGLPGPSGPLGDSGPQGLKGVKGNPGNIRDQPRPAFSAIRQNPMTLGNVVIFDKVLTNQESPYQNHTGRFICAVPGFYYFNFQVISKWDLCLFIKSSSGGQPRDSLSFSNTNNKGLFQVLAGGTVLQLRRGDEVWIEKDPAKGRIYQGTEADSIFSGFLIFPSA

SEQ ID NO: 15 - protein, 246 aa, Mus musculus
MVVGPSCQPPCGLCLLLLFLLALPLRSQASAGCYGIPGMPGMPGAPGKDGHDGLQGPKGEPGIPAVPGTRGPKGQKGEPGMPGHRGKNGPRGTSGLPGDPGPRGPPGEPGVEGRYKQKHQSVFTVTRQTTQYPEANALVRFNSVVTNPQGHYNPSTGKFTCEVPGLYYFVYYTSHTANLCVHLNLNLARVASFCDHMFNSKQVSSGGVLLRLQRGDEVWLSVNDYNGMVGIEGSNSVFSGFLLFPD

SEQ ID NO: 16 - protein, 31 aa, Homo sapiens
GLFQVVSGGMVLQLQQGDQVWVEKDPKKGHI

SEQ ID NO: 17 - protein, 26 aa, Homo sapiens
GLFQVVSGGMVLQLQQGDQVWVEKDP

SEQ ID NO: 18 - protein, 20 aa, Homo sapiens
SGGMVLQLQQGDQVWVEKDP

SEQ ID NO: 19 - protein, 18 aa, Homo sapiens
SGGMVLQLQQGDQVWVEK

SEQ ID NO: 20 - protein, 23 aa, Homo sapiens
WLAVNDYYDMVGIQGSDSVFSGF

SEQ ID NO: 21 - protein, 16 aa, Homo sapiens
YDMVGIQGSDSVFSGF

SEQ ID NO: 22 - protein, 8 aa, Homo sapiens
YDMVGIQG

SEQ ID NO: 23 - protein, 23 aa, Homo sapiens
HTANLCVLLYRSGVKVVTFCGHT

SEQ ID NO: 24 - protein, 9 aa, Homo sapiens
RSGVKVVTF

SEQ ID NO: 25 - protein, 24 aa, Homo sapiens
GLFQVVSGGMVLQLQQGDQVWVEK

SEQ ID NO: 26 - protein, 12 aa, Homo sapiens
FQVVSGGMVLQL